European Patent Application EP 4 640 224 A1, published October 29, 2025. Title: 나트륨 포도당 운반체-2 저해제 및 안지오텐신 Ⅱ 수용체 차단제를 함유하는 비알코올성 지방간 질환 예방 또는 치료용 약학적 조성물. Applicant: 주식회사 티에치팜. The sequence listing filed with the application follows.

SEQUENCE LISTING (6 sequences)

SEQ ID NO: 1 - DNA, 22 bp, synthetic construct
  source 1..22: mol_type = other DNA
tcctgagccatgcagaatttac

SEQ ID NO: 2 - DNA, 20 bp, synthetic construct
  source 1..20: mol_type = other DNA
agtctaaggcctcgctggtg

SEQ ID NO: 3 - DNA, 25 bp, synthetic construct
  source 1..25: mol_type = other DNA
attccattcacaagaacagatccag

SEQ ID NO: 4 - DNA, 25 bp, synthetic construct
  source 1..25: mol_type = other DNA
tttatctccacagacacgacattca

SEQ ID NO: 5 - DNA, 18 bp, synthetic construct
  source 1..18: mol_type = other DNA
cctggcacccagcacaat

SEQ ID NO: 6 - DNA, 22 bp, synthetic construct
  source 1..22: mol_type = other DNA
gccgatccacacacggagtact